European Patent Specification EP 4 006 170 B1, published February 11, 2026. Title: CRISPR MULTI-TARGET DETECTION METHOD AND TEST KIT THEREFOR. Applicant: SHANGHAI TOLO BIOTECHNOLOGY COMPANY LIMITED. Application PCT/CN2020/104588. The sequence listing filed with the application follows.

SEQUENCE LISTING (34 sequences)

SEQ ID NO: 1 - DNA, 54 bp, Artificial sequence
  Probe sequence
gaauuucuacuguuguagaucugaugguccaugucuguuacucctctaacagac

SEQ ID NO: 2 - DNA, 55 bp, Artificial sequence
  Probe sequence
aauuucuacuguuguagauucucugugcauggccuguaauuuccttattacaggc

SEQ ID NO: 3 - DNA, 20 bp, Artificial sequence
  Primer sequence
gtgaacgttcccttagcact

SEQ ID NO: 4 - DNA, 19 bp, Artificial sequence
  Primer sequence
gggagggcagaactagtcc

SEQ ID NO: 5 - DNA, 41 bp, Artificial sequence
  Primer sequence
cgccacttgacaggcgagtaactgccacttattgggtcagc

SEQ ID NO: 6 - DNA, 39 bp, Artificial sequence
  Primer sequence
gcgtgttccccagagtgacttagcagcttcctcctcctt

SEQ ID NO: 7 - DNA, 22 bp, Artificial sequence
  Primer sequence
aggaaacattaacgtactgatg

SEQ ID NO: 8 - DNA, 21 bp, Artificial sequence
  Primer sequence
ttccttttatttcccttcagc

SEQ ID NO: 9 - DNA, 19 bp, Artificial sequence
  Primer sequence
tctctgtgcatggcctgta

SEQ ID NO: 10 - DNA, 20 bp, Artificial sequence
  Primer sequence
aacagtaaaggcaacgtcca

SEQ ID NO: 11 - DNA, 40 bp, Artificial sequence
  Primer sequence
gcagctgggataccagtggaagtgcctcctggaagaatgg

SEQ ID NO: 12 - DNA, 40 bp, Artificial sequence
  Primer sequence
tctctagagccatcttgcgcctgaagcgacccatgaacgc

SEQ ID NO: 13 - DNA, 22 bp, Artificial sequence
  Primer sequence
tgcttactgaagccgaaaaatg

SEQ ID NO: 14 - DNA, 21 bp, Artificial sequence
  Primer sequence
tgatcgcgagaccacacgatg

SEQ ID NO: 15 - DNA, 16 bp, Artificial sequence
  Primer sequence
cgccgccaactacggt

SEQ ID NO: 16 - DNA, 16 bp, Artificial sequence
  Primer sequence
cggcgctggacgagat

SEQ ID NO: 17 - DNA, 39 bp, Artificial sequence
  Primer sequence
gcatctggccacctcgatgccttacggtgcccgcaaagt

SEQ ID NO: 18 - DNA, 38 bp, Artificial sequence
  Primer sequence
acggctgatgaccaaactcggcggctgtggccggatca

SEQ ID NO: 19 - DNA, 18 bp, Artificial sequence
  Primer sequence
tcacggttcagggttagc

SEQ ID NO: 20 - DNA, 20 bp, Artificial sequence
  Primer sequence
aagcccgcaggaccacgatc

SEQ ID NO: 21 - DNA, 53 bp, Artificial sequence
  Probe sequence
aauuucuacuguuguagauugaacuuuauuggcgguauuucggctaataccgc

SEQ ID NO: 22 - DNA, 53 bp, Artificial sequence
  Probe sequence
aauuucuacuguuguagaucacuaccaccaaauaacuggucggctccagttat

SEQ ID NO: 23 - DNA, 97 bp, Artificial sequence
  Synthetic Cas12b_tracrRNA
tttttgagaagctcaacgggctttgccacctggaaagtggccattggcacacccgttgaaaaattctgtcctctagaccctatagtgagtcgtatta

SEQ ID NO: 24 - DNA, 25 bp, Artificial sequence
  T7-crRNA-F primer
gaaattaatacgactcactataggg

SEQ ID NO: 25 - DNA, 20 bp, Artificial sequence
  Primer sequence
tgtcaccgtggtccagttta

SEQ ID NO: 26 - DNA, 20 bp, Artificial sequence
  Primer sequence
cgacaagaccatcaccaatg

SEQ ID NO: 27 - DNA, 23 bp, Artificial sequence
  Primer sequence
gatgggaacgattatatcgaagg

SEQ ID NO: 28 - DNA, 24 bp, Artificial sequence
  Primer sequence
cctgacagaatattataagctccg

SEQ ID NO: 29 - DNA, 50 bp, Artificial sequence
  Probe sequence
gacgaaugaaggaaugcaacugaacuuuauuggcgguauutttaccgcca

SEQ ID NO: 30 - DNA, 51 bp, Artificial sequence
  Probe sequence
gacgaaugaaggaaugcaaccacuaccaccaaauaacuggggtgttatttg

SEQ ID NO: 31 - DNA, 24 bp, Artificial sequence
  Cas14a-tracr-R primer
aaatgaatttgtttcgagggttac

SEQ ID NO: 32 - DNA, 168 bp, Artificial sequence
  Synthetic Cas14a1 tracrRNA sequence
gaaattaatacgactcactatagggcttcactgataaagtggagaaccgcttcaccaaaagctgtcccttaggggattagaacttgagtgaaggtgggctgcttgcatcagcctaatgtcgagaagtgctttcttcggaaagtaaccctcgaaacaaattcatttttc

SEQ ID NO: 33 - DNA, 20 bp, Artificial sequence
  Primer sequence
cgacaagaccatcaccaatg

SEQ ID NO: 34 - DNA, 20 bp, Artificial sequence
  Primer sequence
cagtagggaagcgaacagag